European Patent Specification EP 4 192 851 B1, published January 29, 2025. Title: Improved N-terminal capping modules of ankyrin repeat domains. Applicant: Athebio AG. The sequence listing filed with the application follows.

SEQUENCE LISTING (133 sequences)

SEQ ID NO: 1 - protein, 30 aa, Artificial Sequence
  Synthetic Construct
DLGKKLLEAARAGQDDEVRELLKAGADVNA

SEQ ID NO: 2 - protein, 30 aa, Artificial Sequence
  Synthetic Construct
DLGKKLLEAARAGQDDEVRILLKAGADVNA

SEQ ID NO: 3 - protein, 30 aa, Artificial Sequence
  Synthetic Construct
DLGKKLLEAARAGQDDEVRILMANGADVNA

SEQ ID NO: 4 - protein, 30 aa, Artificial Sequence
  Synthetic Construct
DLDKKLLEAARAGQDDEVRILMANGADVNA

SEQ ID NO: 5 - protein, 30 aa, Artificial Sequence
  Synthetic Construct
DLGKKLLEAARAGQDDEVRILIANGAPFTT

SEQ ID NO: 6 - protein, 30 aa, Artificial Sequence
  Synthetic Construct
DLGKKLLEAARAGQDDEVRELTKAGADVNA

SEQ ID NO: 7 - protein, 30 aa, Artificial Sequence
  Synthetic Construct
  VARIANT 15: Xaa can be any naturally occuring amino acid
DLGKKLLEAARAGQXDEVRILMANGADVNA

SEQ ID NO: 8 - protein, 30 aa, Artificial Sequence
  Synthetic Construct
  VARIANT 15: Xaa can be any naturally occuring amino acid
DLGKKLLEAARAGQXDEVRELLKAGADVNA

SEQ ID NO: 9 - protein, 30 aa, Artificial Sequence
  Synthetic Construct
  VARIANT 15: Xaa can be any naturally occuring amino acid
DLDKKLLEAARAGQXDEVRELTKAGADVNA

SEQ ID NO: 10 - protein, 30 aa, Artificial Sequence
  Synthetic Construct
  VARIANT 15: Xaa can be any naturally occuring amino acid
DLGKKLLEAARAGQXDEVRELIKAGADVNA

SEQ ID NO: 11 - protein, 30 aa, Artificial Sequence
  Synthetic Construct
  VARIANT 15: Xaa can be any naturally occuring amino acid
DLDKKLLEAAAAGQXDAVRELLKAGADVNA

SEQ ID NO: 12 - protein, 30 aa, Artificial Sequence
  Synthetic Construct
  VARIANT 15: Xaa can be any naturally occuring amino acid
DLAKKLLEAAAAGQXDAVRELVKAGADVNA

SEQ ID NO: 13 - protein, 30 aa, Artificial Sequence
  Synthetic Construct
  VARIANT 15: Xaa can be any naturally occuring amino acid
DLGKKLLEAAAAGQXDAVRELIKAGADVNA

SEQ ID NO: 14 - protein, 30 aa, Artificial Sequence
  Synthetic Construct
  VARIANT 15: Xaa can be any naturally occuring amino acid
DLAKKLLEAAAAGQXDAVRELAKAGADVNA

SEQ ID NO: 15 - protein, 30 aa, Artificial Sequence
  Synthetic Construct
  VARIANT 15: Xaa can be any naturally occuring amino acid
DLAKKLLAAAAAGQXEAVEQLLKAGADVNA

SEQ ID NO: 16 - protein, 30 aa, Artificial Sequence
  Synthetic Construct
  VARIANT 15: Xaa can be any naturally occuring amino acid
DLGKKLLAAAAAGQXEAVEQLIKAGADVNA

SEQ ID NO: 17 - protein, 30 aa, Artificial Sequence
  Synthetic Construct
DLGKKLLEAARAGQIDEVRILMANGADVNA

SEQ ID NO: 18 - protein, 30 aa, Artificial Sequence
  Synthetic Construct
DLGKKLLEAARAGQIDEVRELLKAGADVNA

SEQ ID NO: 19 - protein, 30 aa, Artificial Sequence
  Synthetic Construct
DLDKKLLEAARAGQIDEVRELTKAGADVNA

SEQ ID NO: 20 - protein, 30 aa, Artificial Sequence
  Synthetic Construct
DLGKKLLEAARAGQIDEVRELIKAGADVNA

SEQ ID NO: 21 - protein, 30 aa, Artificial Sequence
  Synthetic Construct
DLDKKLLEAAAAGQIDAVRELLKAGADVNA

SEQ ID NO: 22 - protein, 30 aa, Artificial Sequence
  Synthetic Construct
DLAKKLLEAAAAGQIDAVRELVKAGADVNA

SEQ ID NO: 23 - protein, 30 aa, Artificial Sequence
  Synthetic Construct
DLGKKLLEAAAAGQIDAVRELIKAGADVNA

SEQ ID NO: 24 - protein, 30 aa, Artificial Sequence
  Synthetic Construct
DLAKKLLEAAAAGQIDAVRELAKAGADVNA

SEQ ID NO: 25 - protein, 30 aa, Artificial Sequence
  Synthetic Construct
DLAKKLLAAAAAGQIEAVEQLLKAGADVNA

SEQ ID NO: 26 - protein, 30 aa, Artificial Sequence
  Synthetic Construct
DLGKKLLAAAAAGQIEAVEQLIKAGADVNA

SEQ ID NO: 27 - protein, 30 aa, Artificial Sequence
  Synthetic Construct
DLGKKLLEAARAGQTDEVRILMANGADVNA

SEQ ID NO: 28 - protein, 30 aa, Artificial Sequence
  Synthetic Construct
DLGKKLLEAARAGQTDEVRELLKAGADVNA

SEQ ID NO: 29 - protein, 30 aa, Artificial Sequence
  Synthetic Construct
DLDKKLLEAARAGQTDEVRELTKAGADVNA

SEQ ID NO: 30 - protein, 30 aa, Artificial Sequence
  Synthetic Construct
DLGKKLLEAARAGQTDEVRELIKAGADVNA

SEQ ID NO: 31 - protein, 30 aa, Artificial Sequence
  Synthetic Construct
DLDKKLLEAAAAGQTDAVRELLKAGADVNA

SEQ ID NO: 32 - protein, 30 aa, Artificial Sequence
  Synthetic Construct
DLAKKLLEAAAAGQTDAVRELVKAGADVNA

SEQ ID NO: 33 - protein, 30 aa, Artificial Sequence
  Synthetic Construct
DLGKKLLEAAAAGQTDAVRELIKAGADVNA

SEQ ID NO: 34 - protein, 30 aa, Artificial Sequence
  Synthetic Construct
DLAKKLLEAAAAGQTDAVRELAKAGADVNA

SEQ ID NO: 35 - protein, 30 aa, Artificial Sequence
  Synthetic Construct
DLAKKLLAAAAAGQTEAVEQLLKAGADVNA

SEQ ID NO: 36 - protein, 30 aa, Artificial Sequence
  Synthetic Construct
DLGKKLLAAAAAGQTEAVEQLIKAGADVNA

SEQ ID NO: 37 - protein, 30 aa, Artificial Sequence
  Synthetic Construct
DLGKKLLEAARAGQADEVRILMANGADVNA

SEQ ID NO: 38 - protein, 30 aa, Artificial Sequence
  Synthetic Construct
DLGKKLLEAARAGQADEVRELLKAGADVNA

SEQ ID NO: 39 - protein, 30 aa, Artificial Sequence
  Synthetic Construct
DLDKKLLEAARAGQADEVRELTKAGADVNA

SEQ ID NO: 40 - protein, 30 aa, Artificial Sequence
  Synthetic Construct
DLGKKLLEAARAGQADEVRELIKAGADVNA

SEQ ID NO: 41 - protein, 30 aa, Artificial Sequence
  Synthetic Construct
DLDKKLLEAAAAGQADAVRELLKAGADVNA

SEQ ID NO: 42 - protein, 30 aa, Artificial Sequence
  Synthetic Construct
DLAKKLLEAAAAGQADAVRELVKAGADVNA

SEQ ID NO: 43 - protein, 30 aa, Artificial Sequence
  Synthetic Construct
DLGKKLLEAAAAGQADAVRELIKAGADVNA

SEQ ID NO: 44 - protein, 30 aa, Artificial Sequence
  Synthetic Construct
DLAKKLLEAAAAGQADAVRELAKAGADVNA

SEQ ID NO: 45 - protein, 30 aa, Artificial Sequence
  Synthetic Construct
DLAKKLLAAAAAGQAEAVEQLLKAGADVNA

SEQ ID NO: 46 - protein, 30 aa, Artificial Sequence
  Synthetic Construct
DLGKKLLAAAAAGQAEAVEQLIKAGADVNA

SEQ ID NO: 47 - protein, 30 aa, Artificial Sequence
  Synthetic Construct
DLGKKLLEAARAGQVDEVRILMANGADVNA

SEQ ID NO: 48 - protein, 30 aa, Artificial Sequence
  Synthetic Construct
DLGKKLLEAARAGQVDEVRELLKAGADVNA

SEQ ID NO: 49 - protein, 30 aa, Artificial Sequence
  Synthetic Construct
DLDKKLLEAARAGQVDEVRELTKAGADVNA

SEQ ID NO: 50 - protein, 30 aa, Artificial Sequence
  Synthetic Construct
DLGKKLLEAARAGQVDEVRELIKAGADVNA

SEQ ID NO: 51 - protein, 30 aa, Artificial Sequence
  Synthetic Construct
DLDKKLLEAAAAGQVDAVRELLKAGADVNA

SEQ ID NO: 52 - protein, 30 aa, Artificial Sequence
  Synthetic Construct
DLAKKLLEAAAAGQVDAVRELVKAGADVNA

SEQ ID NO: 53 - protein, 30 aa, Artificial Sequence
  Synthetic Construct
DLGKKLLEAAAAGQVDAVRELIKAGADVNA

SEQ ID NO: 54 - protein, 30 aa, Artificial Sequence
  Synthetic Construct
DLAKKLLEAAAAGQVDAVRELAKAGADVNA

SEQ ID NO: 55 - protein, 30 aa, Artificial Sequence
  Synthetic Construct
DLAKKLLAAAAAGQVEAVEQLLKAGADVNA

SEQ ID NO: 56 - protein, 30 aa, Artificial Sequence
  Synthetic Construct
DLGKKLLAAAAAGQVEAVEQLIKAGADVNA

SEQ ID NO: 57 - protein, 30 aa, Artificial Sequence
  Synthetic Construct
DLGKKLLEAARAGQLDEVRILMANGADVNA

SEQ ID NO: 58 - protein, 30 aa, Artificial Sequence
  Synthetic Construct
DLGKKLLEAARAGQLDEVRELLKAGADVNA

SEQ ID NO: 59 - protein, 30 aa, Artificial Sequence
  Synthetic Construct
DLDKKLLEAARAGQLDEVRELTKAGADVNA

SEQ ID NO: 60 - protein, 30 aa, Artificial Sequence
  Synthetic Construct
DLGKKLLEAARAGQLDEVRELIKAGADVNA

SEQ ID NO: 61 - protein, 30 aa, Artificial Sequence
  Synthetic Construct
DLDKKLLEAAAAGQLDAVRELLKAGADVNA

SEQ ID NO: 62 - protein, 30 aa, Artificial Sequence
  Synthetic Construct
DLAKKLLEAAAAGQLDAVRELVKAGADVNA

SEQ ID NO: 63 - protein, 30 aa, Artificial Sequence
  Synthetic Construct
DLGKKLLEAAAAGQLDAVRELIKAGADVNA

SEQ ID NO: 64 - protein, 30 aa, Artificial Sequence
  Synthetic Construct
DLAKKLLEAAAAGQLDAVRELAKAGADVNA

SEQ ID NO: 65 - protein, 30 aa, Artificial Sequence
  Synthetic Construct
DLAKKLLAAAAAGQLEAVEQLLKAGADVNA

SEQ ID NO: 66 - protein, 30 aa, Artificial Sequence
  Synthetic Construct
DLGKKLLAAAAAGQLEAVEQLIKAGADVNA

SEQ ID NO: 67 - protein, 30 aa, Artificial Sequence
  Synthetic Construct
DLGKKLLEAARAGQMDEVRILMANGADVNA

SEQ ID NO: 68 - protein, 30 aa, Artificial Sequence
  Synthetic Construct
DLGKKLLEAARAGQMDEVRELLKAGADVNA

SEQ ID NO: 69 - protein, 30 aa, Artificial Sequence
  Synthetic Construct
DLDKKLLEAARAGQMDEVRELTKAGADVNA

SEQ ID NO: 70 - protein, 30 aa, Artificial Sequence
  Synthetic Construct
DLGKKLLEAARAGQMDEVRELIKAGADVNA

SEQ ID NO: 71 - protein, 30 aa, Artificial Sequence
  Synthetic Construct
DLDKKLLEAAAAGQMDAVRELLKAGADVNA

SEQ ID NO: 72 - protein, 30 aa, Artificial Sequence
  Synthetic Construct
DLAKKLLEAAAAGQMDAVRELVKAGADVNA

SEQ ID NO: 73 - protein, 30 aa, Artificial Sequence
  Synthetic Construct
DLGKKLLEAAAAGQMDAVRELIKAGADVNA

SEQ ID NO: 74 - protein, 30 aa, Artificial Sequence
  Synthetic Construct
DLAKKLLEAAAAGQMDAVRELAKAGADVNA

SEQ ID NO: 75 - protein, 30 aa, Artificial Sequence
  Synthetic Construct
DLAKKLLAAAAAGQMEAVEQLLKAGADVNA

SEQ ID NO: 76 - protein, 30 aa, Artificial Sequence
  Synthetic Construct
DLGKKLLAAAAAGQMEAVEQLIKAGADVNA

SEQ ID NO: 77 - protein, 33 aa, Artificial Sequence
  Synthetic Construct
  VARIANT 1: Xaa can be any naturally occuring amino acid
  VARIANT 3: Xaa can be any naturally occuring amino acid
  VARIANT 4: Xaa can be any naturally occuring amino acid
  VARIANT 6: Xaa can be any naturally occuring amino acid
  VARIANT 13: Xaa can be any naturally occuring amino acid
  VARIANT 14: Xaa can be any naturally occuring amino acid
  VARIANT 15: Xaa can be any naturally occuring amino acid
  VARIANT 17: Xaa can be any naturally occuring amino acid
  VARIANT 18: Xaa can be any naturally occuring amino acid
  VARIANT 19: Xaa can be any naturally occuring amino acid
  VARIANT 22: Xaa can be any naturally occuring amino acid
  VARIANT 26: Xaa can be any naturally occuring amino acid
  VARIANT 27: Xaa can be any naturally occuring amino acid
XDXXGXTPLHLAXXXGXXXVVXLLLXXGADVNA

SEQ ID NO: 78 - protein, 33 aa, Artificial Sequence
  Synthetic Construct
  VARIANT 1: Xaa can be any naturally occuring amino acid
  VARIANT 3: Xaa can be any naturally occuring amino acid
  VARIANT 4: Xaa can be any naturally occuring amino acid
  VARIANT 6: Xaa can be any naturally occuring amino acid
  VARIANT 14: Xaa can be any naturally occuring amino acid
  VARIANT 15: Xaa can be any naturally occuring amino acid
  VARIANT 27: Xaa can be any naturally occuring amino acid
XDXXGXTPLHLAAXXGHLEIVEVLLKXGADVNA

SEQ ID NO: 79 - protein, 33 aa, Artificial Sequence
  Synthetic Construct
  VARIANT 2: Xaa can be any naturally occuring amino acid
  VARIANT 3: Xaa can be any naturally occuring amino acid
  VARIANT 4: Xaa can be any naturally occuring amino acid
  VARIANT 6: Xaa can be any naturally occuring amino acid
  VARIANT 11: Xaa can be any naturally occuring amino acid
  VARIANT 14: Xaa can be any naturally occuring amino acid
  VARIANT 15: Xaa can be any naturally occuring amino acid
  VARIANT 27: Xaa can be any naturally occuring amino acid
SXXXGXTPLHXAAXXGHLEIVDVLLAXGADVNA

SEQ ID NO: 80 - protein, 33 aa, Artificial Sequence
  Synthetic Construct
  VARIANT 1: Xaa can be any naturally occuring amino acid
  VARIANT 3: Xaa can be any naturally occuring amino acid
  VARIANT 4: Xaa can be any naturally occuring amino acid
  VARIANT 6: Xaa can be any naturally occuring amino acid
  VARIANT 14: Xaa can be any naturally occuring amino acid
  VARIANT 15: Xaa can be any naturally occuring amino acid
XDXXGXTPLHLAAXXGHLEIVEVLLKNGADVNA

SEQ ID NO: 81 - protein, 33 aa, Artificial Sequence
  Synthetic Construct
  VARIANT 3: Xaa can be any naturally occuring amino acid
  VARIANT 4: Xaa can be any naturally occuring amino acid
  VARIANT 6: Xaa can be any naturally occuring amino acid
  VARIANT 14: Xaa can be any naturally occuring amino acid
  VARIANT 15: Xaa can be any naturally occuring amino acid
KDXXGXTPLHLAAXXGHLEIVEVLLKAGADVNA

SEQ ID NO: 82 - protein, 33 aa, Artificial Sequence
  Synthetic Construct
  VARIANT 1: Xaa can be any naturally occuring amino acid
  VARIANT 3: Xaa can be any naturally occuring amino acid
  VARIANT 4: Xaa can be any naturally occuring amino acid
  VARIANT 6: Xaa can be any naturally occuring amino acid
  VARIANT 11: Xaa can be any naturally occuring amino acid
  VARIANT 14: Xaa can be any naturally occuring amino acid
  VARIANT 15: Xaa can be any naturally occuring amino acid
  VARIANT 27: Xaa can be any naturally occuring amino acid
XDXXGXTPLHXAAXXGHLEVVKLLLEXGADVNA

SEQ ID NO: 83 - protein, 28 aa, Artificial Sequence
  Synthetic Construct
QDKFGKTAFDISIDNGNEDLAEILQKLN

SEQ ID NO: 84 - protein, 28 aa, Artificial Sequence
  Synthetic Construct
QDKFGKTAFDISIDNGNEDLAEILQKAA

SEQ ID NO: 85 - protein, 28 aa, Artificial Sequence
  Synthetic Construct
QDKFGKTPFDLAIDNGNEDIAEVLQKAA

SEQ ID NO: 86 - protein, 28 aa, Artificial Sequence
  Synthetic Construct
QDKFGKTPFDLAIREGHEDIAEVLQKAA

SEQ ID NO: 87 - protein, 28 aa, Artificial Sequence
  Synthetic Construct
QDKSGKTPADLAADAGHEDIAEVLQKAA

SEQ ID NO: 88 - protein, 28 aa, Artificial Sequence
  Synthetic Construct
QDSAGKTPADLAADAGHEEIAEVLQKAA

SEQ ID NO: 89 - protein, 28 aa, Artificial Sequence
  Synthetic Construct
QDKAGLTPADLAADAGHEEIAEVLQKAA

SEQ ID NO: 90 - protein, 28 aa, Artificial Sequence
  Synthetic Construct
QDSLGKTPADLAALAGHEEIAEVLQKAA

SEQ ID NO: 91 - protein, 28 aa, Artificial Sequence
  Synthetic Construct
QDKAGQTPADLAADAGHEEIAEVLQKAA

SEQ ID NO: 92 - protein, 28 aa, Artificial Sequence
  Synthetic Construct
  VARIANT 3: Xaa can be any naturally occuring amino acid
  VARIANT 4: Xaa can be any naturally occuring amino acid
  VARIANT 6: Xaa can be any naturally occuring amino acid
  VARIANT 14: Xaa can be any naturally occuring amino acid
QDXXGXTPADLAAXAGHEEIAEVLQKAA

SEQ ID NO: 93 - protein, 103 aa, Artificial Sequence
  Synthetic Construct
MRGSHHHHHHGSDLGKKLLEAARAGQDDEVRILMANGADVNAKDKDGYTPLHLAAREGHLEIVEVLLKAGADVNAQDKFGKTAFDISIDNGNEDLAEILQKLN

SEQ ID NO: 94 - protein, 103 aa, Artificial Sequence
  Synthetic Construct
MRGSHHHHHHGSDLGKKLLEAARAGQLDEVRILMANGADVNAKDKDGYTPLHLAAREGHLEIVEVLLKAGADVNAQDKFGKTAFDISIDNGNEDLAEILQKLN

SEQ ID NO: 95 - protein, 103 aa, Artificial Sequence
  Synthetic Construct
MRGSHHHHHHGSDLGKKLLEAARAGQDDEVRELLKAGADVNAKDKDGYTPLHLAAREGHLEIVEVLLKAGADVNAQDKFGKTAFDISIDNGNEDLAEILQKLN

SEQ ID NO: 96 - protein, 103 aa, Artificial Sequence
  Synthetic Construct
MRGSHHHHHHGSDLGKKLLEAARAGQLDEVRELLKAGADVNAKDKDGYTPLHLAAREGHLEIVEVLLKAGADVNAQDKFGKTAFDISIDNGNEDLAEILQKLN

SEQ ID NO: 97 - protein, 103 aa, Artificial Sequence
  Synthetic Construct
MRGSHHHHHHGSDLGKKLLEAARAGQMDEVRELLKAGADVNAKDKDGYTPLHLAAREGHLEIVEVLLKAGADVNAQDKFGKTAFDISIDNGNEDLAEILQKLN

SEQ ID NO: 98 - protein, 103 aa, Artificial Sequence
  Synthetic Construct
MRGSHHHHHHGSDLGKKLLEAARAGQIDEVRELLKAGADVNAKDKDGYTPLHLAAREGHLEIVEVLLKAGADVNAQDKFGKTAFDISIDNGNEDLAEILQKLN

SEQ ID NO: 99 - protein, 103 aa, Artificial Sequence
  Synthetic Construct
MRGSHHHHHHGSDLGKKLLEAARAGQTDEVRELLKAGADVNAKDKDGYTPLHLAAREGHLEIVEVLLKAGADVNAQDKFGKTAFDISIDNGNEDLAEILQKLN

SEQ ID NO: 100 - protein, 103 aa, Artificial Sequence
  Synthetic Construct
MRGSHHHHHHGSDLGKKLLEAARAGQADEVRELLKAGADVNAKDKDGYTPLHLAAREGHLEIVEVLLKAGADVNAQDKFGKTAFDISIDNGNEDLAEILQKLN

SEQ ID NO: 101 - protein, 103 aa, Artificial Sequence
  Synthetic Construct
MRGSHHHHHHGSDLGKKLLEAARAGQVDEVRELLKAGADVNAKDKDGYTPLHLAAREGHLEIVEVLLKAGADVNAQDKFGKTAFDISIDNGNEDLAEILQKLN

SEQ ID NO: 102 - protein, 103 aa, Artificial Sequence
  Synthetic Construct
MRGSHHHHHHGSDLGKKLLEAARAGQSDEVRELLKAGADVNAKDKDGYTPLHLAAREGHLEIVEVLLKAGADVNAQDKFGKTAFDISIDNGNEDLAEILQKLN

SEQ ID NO: 103 - protein, 103 aa, Artificial Sequence
  Synthetic Construct
MRGSHHHHHHGSDLGKKLLEAARAGQNDEVRELLKAGADVNAKDKDGYTPLHLAAREGHLEIVEVLLKAGADVNAQDKFGKTAFDISIDNGNEDLAEILQKLN

SEQ ID NO: 104 - protein, 103 aa, Artificial Sequence
  Synthetic Construct
MRGSHHHHHHGSDLGKKLLEAARAGQQDEVRELLKAGADVNAKDKDGYTPLHLAAREGHLEIVEVLLKAGADVNAQDKFGKTAFDISIDNGNEDLAEILQKLN

SEQ ID NO: 105 - protein, 103 aa, Artificial Sequence
  Synthetic Construct
MRGSHHHHHHGSDLGKKLLEAARAGQKDEVRELLKAGADVNAKDKDGYTPLHLAAREGHLEIVEVLLKAGADVNAQDKFGKTAFDISIDNGNEDLAEILQKLN

SEQ ID NO: 106 - protein, 103 aa, Artificial Sequence
  Synthetic Construct
MRGSHHHHHHGSDLGKKLLEAARAGQRDEVRELLKAGADVNAKDKDGYTPLHLAAREGHLEIVEVLLKAGADVNAQDKFGKTAFDISIDNGNEDLAEILQKLN

SEQ ID NO: 107 - protein, 103 aa, Artificial Sequence
  Synthetic Construct
MRGSHHHHHHGSDLGKKLLEAARAGQEDEVRELLKAGADVNAKDKDGYTPLHLAAREGHLEIVEVLLKAGADVNAQDKFGKTAFDISIDNGNEDLAEILQKLN

SEQ ID NO: 108 - protein, 103 aa, Artificial Sequence
  Synthetic Construct
MRGSHHHHHHDADLAKKLLAAAAAGQDEAVEQLLKAGADVNAKDKDGYTPLHLAAREGHLEIVEVLLKAGADVNAQDKFGKTAFDISIDNGNEDLAEILQKLN

SEQ ID NO: 109 - protein, 103 aa, Artificial Sequence
  Synthetic Construct
MRGSHHHHHHDADLAKKLLAAAAAGQLEAVEQLLKAGADVNAKDKDGYTPLHLAAREGHLEIVEVLLKAGADVNAQDKFGKTAFDISIDNGNEDLAEILQKLN

SEQ ID NO: 110 - protein, 30 aa, Artificial Sequence
  Synthetic Construct
DLGKKLLQAARAGQLDEVRELLKAGADVNA

SEQ ID NO: 111 - protein, 28 aa, Artificial Sequence
  Synthetic construct
QDKSGKTPADLAARAGHQDIAEVLQKAA

SEQ ID NO: 112 - protein, 28 aa, Artificial Sequence
  Synthetic Construct
QDKFGKTAEDLAKDNGNQDIADLLEKAL

SEQ ID NO: 113 - protein, 136 aa, Artificial Sequence
  Synthetic Construct
MRGSHHHHHHGSDLGKKLLEAARAGQDDEVRELLKAGADVNAKDYFSHTPLHLAARNGHLKIVEVLLKAGADVNAKDFAGKTPLHLAANEGHLEIVEVLLKAGADVNAQDIFGKTPADIAADAGHEDIAEVLQKAA

SEQ ID NO: 114 - protein, 136 aa, Artificial Sequence
  Synthetic Construct
MRGSHHHHHHGSDLGKKLLEAARAGQLDEVRELLKAGADVNAKDYFSHTPLHLAARNGHLKIVEVLLKAGADVNAKDFAGKTPLHLAANEGHLEIVEVLLKAGADVNAQDIFGKTPADIAADAGHEDIAEVLQKAA

SEQ ID NO: 115 - protein, 136 aa, Artificial Sequence
  Synthetic Construct
MRGSHHHHHHGSDLGKKLLEAARAGQVDEVRELLKAGADVNAKDYFSHTPLHLAARNGHLKIVEVLLKAGADVNAKDFAGKTPLHLAANEGHLEIVEVLLKAGADVNAQDIFGKTPADIAADAGHEDIAEVLQKAA

SEQ ID NO: 116 - protein, 136 aa, Artificial Sequence
  Synthetic Construct
MRGSHHHHHHGSDLDKKLLEAARAGQDDEVRILMANGADVNARDSTGWTPLHLAAPWGHPEIVEVLLKNGADVNAADFQGWTPLHLAAAVGHLEIVEVLLKYGADVNAQDKFGKTAFDISIDNGNEDLAEILQKAA

SEQ ID NO: 117 - protein, 136 aa, Artificial Sequence
  Synthetic Construct
MRGSHHHHHHGSDLDKKLLEAARAGQLDEVRILMANGADVNARDSTGWTPLHLAAPWGHPEIVEVLLKNGADVNAADFQGWTPLHLAAAVGHLEIVEVLLKYGADVNAQDKFGKTAFDISIDNGNEDLAEILQKAA

SEQ ID NO: 118 - protein, 136 aa, Artificial Sequence
  Synthetic Construct
MRGSHHHHHHGSDLDKKLLEAARAGQVDEVRILMANGADVNARDSTGWTPLHLAAPWGHPEIVEVLLKNGADVNAADFQGWTPLHLAAAVGHLEIVEVLLKYGADVNAQDKFGKTAFDISIDNGNEDLAEILQKAA

SEQ ID NO: 119 - protein, 136 aa, Artificial Sequence
  Synthetic Construct
MRGSHHHHHHGSDLGKKLLEAARAGQDDEVRILMANGADVNAKDEYGLTPLYLATAHGHLEIVEVLLKNGADVNAVDAIGFTPLHLAAFIGHLEIAEVLLKHGADVNAQDKFGKTAFDISIGNGNEDLAEILQKLN

SEQ ID NO: 120 - protein, 136 aa, Artificial Sequence
  Synthetic Construct
MRGSHHHHHHGSDLGKKLLEAARAGQLDEVRILMANGADVNAKDEYGLTPLYLATAHGHLEIVEVLLKNGADVNAVDAIGFTPLHLAAFIGHLEIAEVLLKHGADVNAQDKFGKTAFDISIGNGNEDLAEILQKLN

SEQ ID NO: 121 - protein, 136 aa, Artificial Sequence
  Synthetic Construct
MRGSHHHHHHGSDLGKKLLEAARAGQVDEVRILMANGADVNAKDEYGLTPLYLATAHGHLEIVEVLLKNGADVNAVDAIGFTPLHLAAFIGHLEIAEVLLKHGADVNAQDKFGKTAFDISIGNGNEDLAEILQKLN

SEQ ID NO: 122 - protein, 103 aa, Artificial Sequence; identical to SEQ ID NO: 96
  Synthetic Construct

SEQ ID NO: 123 - protein, 103 aa, Artificial Sequence
  Synthetic Construct
MRGSHHHHHHGSDLGKKLLEAARAGQLDEVRELIKAGADVNAKDKDGYTPLHLAAREGHLEIVEVLLKAGADVNAQDKFGKTAFDISIDNGNEDLAEILQKLN

SEQ ID NO: 124 - protein, 103 aa, Artificial Sequence; identical to SEQ ID NO: 101
  Synthetic Construct

SEQ ID NO: 125 - protein, 103 aa, Artificial Sequence
  Synthetic Construct
MRGSHHHHHHGSDLGKKLLEAARAGQVDEVRELIKAGADVNAKDKDGYTPLHLAAREGHLEIVEVLLKAGADVNAQDKFGKTAFDISIDNGNEDLAEILQKLN

SEQ ID NO: 126 - protein, 103 aa, Artificial Sequence
  Synthetic Construct
MRGSHHHHHHGSDLGKKLLEAARAGQLDEVKELIAAGADVNAKDKDGYTPLHLAAREGHLEIVEVLLKAGADVNAQDKFGKTAFDISIDNGNEDLAEILQKLN

SEQ ID NO: 127 - protein, 103 aa, Artificial Sequence
  Synthetic Construct
MRGSHHHHHHGSDLGKKLLEAAAAGQLDEVKELIAAGADVNAKDKDGYTPLHLAAREGHLEIVEVLLKAGADVNAQDKFGKTAFDISIDNGNEDLAEILQKLN

SEQ ID NO: 128 - protein, 103 aa, Artificial Sequence
  Synthetic Construct
MRGSHHHHHHGSDLGKKLLEAAEAGQLDEVKELIAAGADVNAKDKDGYTPLHLAAREGHLEIVEVLLKAGADVNAQDKFGKTAFDISIDNGNEDLAEILQKLN

SEQ ID NO: 129 - protein, 169 aa, Artificial Sequence
  Synthetic Construct
MRGSHHHHHHGSDLGKKLLQAARAGQLDEVRELLKAGADVNAKDREGITPLHLAAQHGHLEIVEVLLKAGADVNAKDVWGRTPLHLAAQWGHLEIVEVLLKAGADVNAKDLAGATPLHVAALYGHLEIVEVLLKAGADVNAQDKSGKTPADLAARAGHQDIAEVLQKAA

SEQ ID NO: 130 - protein, 169 aa, Artificial Sequence
  Synthetic Construct
MRGSHHHHHHGSDLGKKLLQAARAGQLDEVRELLKLGADVNAKDREGITPLHLAAQHGHLEIVEVLLKAGADVNAKDVWGRTPLHLAAQWGHLEIVEVLLKAGADVNAKDLAGATPLHVAALYGHLEIVEVLLKAGADVNAQDKSGKTPADLAARAGHQDIAEVLQKAA

SEQ ID NO: 131 - protein, 24 aa, Artificial Sequence
  Linker
GSPTPTPTTPTPTPTTPTPTPTGS

SEQ ID NO: 132 - protein, 22 aa, Artificial Sequence
  Linker
GSPTPTPTTPTPTPTTPTPTPT

SEQ ID NO: 133 - protein, 5 aa, Artificial Sequence
  Linker
GGGGS